European Patent Application EP 4 603 099 A1, published August 20, 2025. Title: Anti-influenza virus composition. Applicant: Hokkaido University. Application JP. The sequence listing filed with the application follows.

SEQUENCE LISTING (55 sequences)

SEQ ID NO: 1 - DNA, 20 bp, Artificial
  source 1..20: mol_type = other DNA
gacatggagggaggagatca

SEQ ID NO: 2 - DNA, 20 bp, Artificial
  source 1..20: mol_type = other DNA
tataggctgagctgcctggt

SEQ ID NO: 3 - DNA, 20 bp, Artificial
  source 1..20: mol_type = other DNA
ggactgcagcgtagacgctt

SEQ ID NO: 4 - DNA, 24 bp, Artificial
  source 1..24: mol_type = other DNA
catcctgttgtatatgaggcccat

SEQ ID NO: 5 - DNA, 25 bp, Artificial
  source 1..25: mol_type = other DNA
ggagtatcggatgcttccagaacca

SEQ ID NO: 6 - DNA, 23 bp, Artificial
  source 1..23: mol_type = other DNA
acgaccttctggcacaagaggtt

SEQ ID NO: 7 - DNA, 20 bp, Artificial
  source 1..20: mol_type = other DNA
ttatagtgccggacctggca

SEQ ID NO: 8 - DNA, 20 bp, Artificial
  source 1..20: mol_type = other DNA
cccaagctcccagtgttgtc

SEQ ID NO: 9 - DNA, 20 bp, Artificial
  source 1..20: mol_type = other DNA
ggaggcacaggatgtaatca

SEQ ID NO: 10 - DNA, 20 bp, Artificial
  source 1..20: mol_type = other DNA
cgttagttgcgattccgatg

SEQ ID NO: 11 - DNA, 20 bp, Artificial
  source 1..20: mol_type = other DNA
acacaaggccgacagaccta

SEQ ID NO: 12 - DNA, 20 bp, Artificial
  source 1..20: mol_type = other DNA
atgctgttgcagcaggttgg

SEQ ID NO: 13 - DNA, 20 bp, Artificial
  source 1..20: mol_type = other DNA
gcactcacttggaagtatgc

SEQ ID NO: 14 - DNA, 20 bp, Artificial
  source 1..20: mol_type = other DNA
ttgactcgccttgctcattg

SEQ ID NO: 15 - DNA, 20 bp, Artificial
  source 1..20: mol_type = other DNA
ctgctcgaagacagccacaa

SEQ ID NO: 16 - DNA, 20 bp, Artificial
  source 1..20: mol_type = other DNA
gagccatccggcgatgttac

SEQ ID NO: 17 - DNA, 20 bp, Artificial
  source 1..20: mol_type = other DNA
acggctggtctgactcacat

SEQ ID NO: 18 - DNA, 20 bp, Artificial
  source 1..20: mol_type = other DNA
tccattccggtgcgaacaag

SEQ ID NO: 19 - DNA, 20 bp, Artificial
  source 1..20: mol_type = other DNA
ttggtcagcaagtgcatgtc

SEQ ID NO: 20 - DNA, 20 bp, Artificial
  source 1..20: mol_type = other DNA
acagccactgctccattatc

SEQ ID NO: 21 - DNA, 20 bp, Artificial
  source 1..20: mol_type = other DNA
caagcagcagaggccatgga

SEQ ID NO: 22 - DNA, 20 bp, Artificial
  source 1..20: mol_type = other DNA
gaccagcactggagctagga

SEQ ID NO: 23 - DNA, 20 bp, Artificial
  source 1..20: mol_type = other DNA
agcagatagtggagcggatt

SEQ ID NO: 24 - DNA, 20 bp, Artificial
  source 1..20: mol_type = other DNA
gtacagaggccatggtcatt

SEQ ID NO: 25 - DNA, 43 bp, Artificial
  source 1..43: mol_type = other DNA
ggccgtcatggtggcgaatgaatggacggagaacaaggattgc

SEQ ID NO: 26 - DNA, 45 bp, Artificial
  source 1..45: mol_type = other DNA
ccagatcgttcgagtcgtttttttttttttttttctttaattgtc

SEQ ID NO: 27 - DNA, 45 bp, Artificial
  source 1..45: mol_type = other DNA
gctagcttcagctaggcatcagtagaaacaagggtatttttcttt

SEQ ID NO: 28 - DNA, 19 bp, Artificial
  source 1..19: mol_type = other DNA
ggccgtcatggtggcgaat

SEQ ID NO: 29 - DNA, 24 bp, Artificial
  source 1..24: mol_type = other DNA
ctcaatatgagtgcagaccgtgct

SEQ ID NO: 30 - DNA, 18 bp, Artificial
  source 1..18: mol_type = other DNA
cgatcgtgccctcctttg

SEQ ID NO: 31 - DNA, 18 bp, Artificial
  source 1..18: mol_type = other DNA
ccagatcgttcgagtcgt

SEQ ID NO: 32 - DNA, 20 bp, Artificial
  source 1..20: mol_type = other DNA
gctagcttcagctaggcatc

SEQ ID NO: 33 - DNA, 20 bp, Artificial
  source 1..20: mol_type = other DNA
gacgtaaacggccacaagtt

SEQ ID NO: 34 - DNA, 20 bp, Artificial
  source 1..20: mol_type = other DNA
gaacttcagggtcagcttgc

SEQ ID NO: 35 - DNA, 18 bp, Artificial
  source 1..18: mol_type = other DNA
caggtaagtatgcaaaag

SEQ ID NO: 36 - DNA, 18 bp, Artificial
  source 1..18: mol_type = other DNA
atcgcttctcggcaaaag

SEQ ID NO: 37 - DNA, 20 bp, Artificial
  source 1..20: mol_type = other DNA
gtatttcattgccatcatcc

SEQ ID NO: 38 - DNA, 21 bp, Artificial
  source 1..21: mol_type = other DNA
ttttggagcagggagatggaa

SEQ ID NO: 39 - DNA, 21 bp, Artificial
  source 1..21: mol_type = other DNA
ggtactgcaataccaggtcga

SEQ ID NO: 40 - DNA, 20 bp, Artificial
  source 1..20: mol_type = other DNA
aaggtgaaggtcggagtcaa

SEQ ID NO: 41 - DNA, 20 bp, Artificial
  source 1..20: mol_type = other DNA
aatgaaggggtcattgatgg

SEQ ID NO: 42 - DNA, 21 bp, Artificial
  source 1..21: mol_type = other DNA
atgtcgctgtttggagacaca

SEQ ID NO: 43 - DNA, 21 bp, Artificial
  source 1..21: mol_type = other DNA
ttctttcccaccgaaccaaca

SEQ ID NO: 44 - DNA, 20 bp, Artificial
  source 1..20: mol_type = other DNA
cttaagaacagcaggcccag

SEQ ID NO: 45 - DNA, 20 bp, Artificial
  source 1..20: mol_type = other DNA
caggggattctaagggcttc

SEQ ID NO: 46 - DNA, 20 bp, Artificial
  source 1..20: mol_type = other DNA
tggagaaaggatgtcggctt

SEQ ID NO: 47 - DNA, 20 bp, Artificial
  source 1..20: mol_type = other DNA
attgatcactgtccctggca

SEQ ID NO: 48 - DNA, 20 bp, Artificial
  source 1..20: mol_type = other DNA
caggacaagatgctgacgaa

SEQ ID NO: 49 - DNA, 20 bp, Artificial
  source 1..20: mol_type = other DNA
gactttggggtgtttgtgct

SEQ ID NO: 50 - DNA, 20 bp, Artificial
  source 1..20: mol_type = other DNA
ccttggatgtgggcaagagg

SEQ ID NO: 51 - DNA, 20 bp, Artificial
  source 1..20: mol_type = other DNA
tagcaggaatagccccgaag

SEQ ID NO: 52 - DNA, 20 bp, Artificial
  source 1..20: mol_type = other DNA
gcagagtacaaagtgcctgg

SEQ ID NO: 53 - DNA, 20 bp, Artificial
  source 1..20: mol_type = other DNA
cagcattttctccgtctccg

SEQ ID NO: 54 - DNA, 17 bp, Artificial
  source 1..17: mol_type = other DNA
taatacgactcactata

SEQ ID NO: 55 - DNA, 45 bp, Artificial
  source 1..45: mol_type = other DNA
cactttcacttctccctttcagtttccctatagtgagtcgtatta